European Patent Application EP 4 737 481 A2, published May 6, 2026. Title: CHIMERIC ANTIGEN RECEPTOR AND CAR-T CELLS THAT BIND BCMA. Applicant: Max-Delbrück-Centrum für Molekulare Medizin in der Helmholtz-Gemeinschaft. Application EP. The sequence listing filed with the application follows.

SEQUENCE LISTING (94 sequences)

SEQ ID NO: 1 - protein, 8 aa, synthetic construct
  REGION 1..8: note = CDR
GFTFSRYW

SEQ ID NO: 2 - protein, 8 aa, synthetic construct
  REGION 1..8: note = CDR
INPSSSTI

SEQ ID NO: 3 - protein, 13 aa, synthetic construct
  REGION 1..13: note = CDR
ASLYYDYGDAYDY

SEQ ID NO: 4 - protein, 6 aa, synthetic construct
  REGION 1..6: note = CDR
QSVESN

SEQ ID NO: 5 - skipped

SEQ ID NO: 6 - protein, 9 aa, synthetic construct
  REGION 1..9: note = CDR
QQYNNYPLT

SEQ ID NO: 7 - protein, 8 aa, synthetic construct
  REGION 1..8: note = CDR
  REGION 4..5: note = misc_feature - Xaa can be any naturally occurring amino acid
INPXXSTI

SEQ ID NO: 8 - protein, 13 aa, synthetic construct
  REGION 1..13: note = CDR
  SITE 5: note = misc_feature - Xaa can be any naturally occurring amino acid
  SITE 11: note = misc_feature - Xaa can be any naturally occurring amino acid
ASLYXDYGDAXDY

SEQ ID NO: 9 - protein, 6 aa, synthetic construct
  REGION 1..6: note = CDR
  REGION 4..5: note = misc_feature - Xaa can be any naturally occurring amino acid
QSVXXN

SEQ ID NO: 10 - protein, 11 aa, synthetic construct
  REGION 1..11: note = CDR
QQYNNYPLTFG

SEQ ID NO: 11 - protein, 120 aa, synthetic construct
  REGION 1..120: note = VH
EVQLVESGGGLVQPGGSLRLSCAASGFTFSRYWFSWVRQAPGKGLVWVGEINPSSSTINYAPSLKDKFTISRDNAKNTLYLQMNSLRAEDTAVYYCASLYYDYGDAYDYWGQGTLVTVSS

SEQ ID NO: 12 - protein, 107 aa, synthetic construct
  REGION 1..107: note = VL
EIVMTQSPATLSVSPGERATLSCKASQSVESNVAWYQQKPGQAPRALIYSASLRFSGIPARFSGSGSGTEFTLTISSLQSEDFAVYYCQQYNNYPLTFGAGTKLELK

SEQ ID NO: 13 - protein, 18 aa, synthetic construct
  REGION 1..18: note = linker
GSTSGSGKPGSGEGSTKG

SEQ ID NO: 14 - protein, 17 aa, synthetic construct
  REGION 1..17: note = linker
SSGGGGSGGGGSGGGGS

SEQ ID NO: 15 - protein, 234 aa, synthetic construct
  REGION 1..234: note = spacer
PAEPKSPDKTHTCPPCPAPPVAGPSVFLFPPKPKDTLMIARTPEVTCVVVDVSHEDPEVKFNWYVDGVEVHNAKTKPREEQYNSTYRVVSVLTVLHQDWLNGKEYKCKVSNKALPAPIEKTISKAKGQPREPQVYTLPPSRDELTKNQVSLTCLVKGFYPSDIAVEWESNGQPENNYKTTPPVLDSDGSFFLYSKLTVDKSRWQQGNVFSCSVMHEALHNHYTQKSLSLSPGKK

SEQ ID NO: 16 - protein, 235 aa, synthetic construct
  REGION 1..235: note = spacer
PAEPKSPDKTHTCPPCPAPPVAGPSVFLFPPKPKDTLMIARTPEVTCVVVDVSHEDPEVKFNWYVDGVEVHNAKTKPREEQYNSTYRVVSVLTVLHQDWLNGKEYKCKVSNKALPAPIEKTISKAKGQPREPQVYTLPPSRDELTKNQVSLTCLVKGFYPSDIAVEWESNGQPENNYKTTPPVLDSDGSFFLYSKLTVDKSRWQQGNVFSCSVMHEALHNHYTQKSLSSLSPGKK

SEQ ID NO: 17 - protein, 229 aa, synthetic construct
  REGION 1..229: note = spacer
ESKYGPPCPPCPAPEFEGGPSVFLFPPKPKDTLMISRTPEVTCVVVDVSQEDPEVQFNWYVDGVEVHNAKTKPREEQFNSTYRVVSVLTVLHQDWLNGKEYKCKVSNKGLPSSIEKTISKAKGQPREPQVYTLPPSQEEMTKNQVSLTCLVKGFYPSDIAVEWESNGQPENNYKTTPPVLDSDGSFFLYSRLTVDKSRWQEGNVFSCSVMHEALHNHYTQKSLSLSLGK

SEQ ID NO: 18 - protein, 119 aa, synthetic construct
  REGION 1..119: note = spacer
ESKYGPPCPPCPGQPREPQVYTLPPSQEEMTKNQVSLTCLVKGFYPSDIAVEWESNGQPENNYKTTPPVLDSDGSFFLYSRLTVDKSRWQEGNVFSCSVMHEALHNHYTQKSLSLSLGK

SEQ ID NO: 19 - protein, 12 aa, synthetic construct
  REGION 1..12: note = spacer
ESKYGPPCPPCP

SEQ ID NO: 20 - protein, 24 aa, synthetic construct
  REGION 1..24: note = transmembrane
IYIWAPLAGTCGVLLLSLVITLYC

SEQ ID NO: 21 - protein, 27 aa, synthetic construct
  REGION 1..27: note = transmembrane
FWVLVVVGGVLACYSLLVTVAFIIFWV

SEQ ID NO: 22 - protein, 42 aa, synthetic construct
  REGION 1..42: note = intracellular
KRGRKKLLYIFKQPFMRPVQTTQEEDGCSCRFPEEEEGGCEL

SEQ ID NO: 23 - protein, 41 aa, synthetic construct
  REGION 1..41: note = intracellular
RSKRSRLLHSDYMNMTPRRPGPTRKHYQPYAPPRDFAAYRS

SEQ ID NO: 24 - protein, 113 aa, synthetic construct
  REGION 1..113: note = intracellular
LRVKFSRSADAPAYQQGQNQLYNELNLGRREEYDVLDKRRGRDPEMGGKPRRKNPQEGLYNELQKDKMAEAYSEIGMKGERRRGKGHDGLYQGLSTATKDTYDALHMQALPPR

SEQ ID NO: 25 - protein, 5 aa, synthetic construct
  REGION 1..5: note = CDR
RYWFS

SEQ ID NO: 26 - protein, 18 aa, synthetic construct
  REGION 1..18: note = CDR
EINPSSSTINYAPSLKDK

SEQ ID NO: 27 - protein, 13 aa, synthetic construct
  REGION 1..13: note = CDR
SLYYDYGDAYDYW

SEQ ID NO: 28 - protein, 11 aa, synthetic construct
  REGION 1..11: note = CDR
KASQSVESNVA

SEQ ID NO: 29 - protein, 7 aa, synthetic construct
  REGION 1..7: note = CDR
SASLRFS

SEQ ID NO: 30 - protein, 11 aa, synthetic construct
  REGION 1..11: note = CDR
QQYNNYPLTFG

SEQ ID NO: 31 - protein, 53 aa, Homo sapiens
MAGQCSQNEYFDSLLHACIPCQLRCSSNTPPLTCQRYCNASVTNSVKGTNALE

SEQ ID NO: 32 - protein, 56 aa, Homo sapiens
MLQMAGQCSQNEYFDSLLHACIPCQLRCSSNTPPLTCQRYCNASVTNSVKGTNALE

SEQ ID NO: 33 - protein, 20 aa, Homo sapiens
YFDSLLHACIPCQLRCSSNT

SEQ ID NO: 34 - protein, 5 aa, synthetic construct
  REGION 1..5: note = CDR
  SITE 4: note = misc_feature - Xaa can be any naturally occurring amino acid
RYWXS

SEQ ID NO: 35 - protein, 18 aa, synthetic construct
  REGION 1..18: note = CDR
  REGION 5..6: note = misc_feature - Xaa can be any naturally occurring amino acid
EINPXXSTINYAPSLKDK

SEQ ID NO: 36 - protein, 13 aa, synthetic construct
  REGION 1..13: note = CDR
  SITE 4: note = misc_feature - Xaa can be any naturally occurring amino acid
  SITE 10: note = misc_feature - Xaa can be any naturally occurring amino acid
SLYXDYGDAXDYW

SEQ ID NO: 37 - protein, 11 aa, synthetic construct
  REGION 1..11: note = CDR
  REGION 7..8: note = misc_feature - Xaa can be any naturally occurring amino acid
KASQSVXXNVA

SEQ ID NO: 38 - protein, 120 aa, synthetic construct
  REGION 1..120: note = mouse Ab
QVQLQQSGGGLVQPGGSLKLSCAASGIDFSRYWMSWVRRAPGKGLEWIGEINPDSSTINYAPSLKDKFIISRDNAKNTLYLQMSKVRSEDTALYYCASLYYDYGDAMDYWGQGTSVTVSS

SEQ ID NO: 39 - protein, 120 aa, synthetic construct
  REGION 1..120: note = Ab
EVQLVESGGGLVQPGGSLRLSCAASGFTFDDYWMSWVRQAPGKGLEWVGEINPDSSTINYAPSLKGRFTISRDNAKNTLYLQMNSLRAEDTAVYYCASLYYDYGDAMDYWGQGTLVTVSS

SEQ ID NO: 40 - protein, 120 aa, synthetic construct
  REGION 1..120: note = VH
EVQLVESGGGLVQPGGSLRLSCAASGFTFSRYWMSWVRQAPGKGLVWVGEINPDSSTINYAPSLKDKFTISRDNAKNTLYLQMNSLRAEDTAVYYCASLYYDYGDAMDYWGQGTLVTVSS

SEQ ID NO: 41 - protein, 120 aa, synthetic construct
  REGION 1..120: note = VH
  SITE 34: note = misc_feature - Xaa can be any naturally occurring amino acid
  REGION 54..55: note = misc_feature - Xaa can be any naturally occurring amino acid
  SITE 101: note = misc_feature - Xaa can be any naturally occurring amino acid
  SITE 107: note = misc_feature - Xaa can be any naturally occurring amino acid
EVQLVESGGGLVQPGGSLRLSCAASGFTFSRYWXSWVRQAPGKGLVWVGEINPXXSTINYAPSLKDKFTISRDNAKNTLYLQMNSLRAEDTAVYYCASLYXDYGDAXDYWGQGTLVTVSS

SEQ ID NO: 42 - protein, 120 aa, synthetic construct
  REGION 1..120: note = VH
  SITE 33: note = misc_feature - Xaa can be any naturally occurring amino acid
  SITE 35: note = misc_feature - Xaa can be any naturally occurring amino acid
  SITE 47: note = misc_feature - Xaa can be any naturally occurring amino acid
  SITE 50: note = misc_feature - Xaa can be any naturally occurring amino acid
  REGION 99..101: note = misc_feature - Xaa can be any naturally occurring amino acid
  SITE 106: note = misc_feature - Xaa can be any naturally occurring amino acid
EVQLVESGGGLVQPGGSLRLSCAASGFTFSRYXMXWVRQAPGKGLVXVGXINPDSSTINYAPSLKDKFTISRDNAKNTLYLQMNSLRAEDTAVYYCASXXXDYGDXMDYWGQGTLVTVSS

SEQ ID NO: 43 - protein, 120 aa, synthetic construct
  REGION 1..120: note = VH
EVQLVESGGGLVQPGGSLRLSCAASGFTFSRYWISWVRQAPGKGLVWVGEINPNSSTINYAPSLKDKFTISRDNAKNTLYLQMNSLRAEDTAVYYCASLYYDYGDAYDYWGQGTLVTVSS

SEQ ID NO: 44 - protein, 120 aa, synthetic construct
  REGION 1..120: note = VH
EVQLVESGGGLVQPGGSLRLSCAASGFTFSRYWFSWVRQAPGKGLVWVGEINPNSSTINYAPSLKDKFTISRDNAKNTLYLQMNSLRAEDTAVYYCASLYYDYGDAYDYWGQGTLVTVSS

SEQ ID NO: 45 - protein, 120 aa, synthetic construct
  REGION 1..120: note = VH
EVQLVESGGGLVQPGGSLRLSCAASGFTFSRYWISWVRQAPGKGLVWVGEINPSSSTINYAPSLKDKFTISRDNAKNTLYLQMNSLRAEDTAVYYCASLYYDYGDAYDYWGQGTLVTVSS

SEQ ID NO: 46 - protein, 120 aa, synthetic construct; identical to SEQ ID NO: 11
  REGION 1..120: note = VH

SEQ ID NO: 47 - protein, 108 aa, synthetic construct
  REGION 1..108: note = VL
DIVMTQSQRFMTTSVGDRVSVTCKASQSVDSNVAWYQQKPRQSPKALIFSASLRFSGVPARFTGSGSGTDFTLTISNLQSEDLAEYFCQQYNNYPLTFGAGTKLELKR

SEQ ID NO: 48 - protein, 108 aa, synthetic construct
  REGION 1..108: note = VL
DIVMTQSPATLSVSVGDEVTLTCKASQSVDSNVAWYQQKPGQAPKLLIYSDDLRFSGVPARFSGSGSGTDFTLTISSLQSEDFAVYYCQQYNNYPLTFGAGTKLELKR

SEQ ID NO: 49 - protein, 108 aa, synthetic construct
  REGION 1..108: note = VL
EIVMTQSPATLSVSPGERATLSCKASQSVDSNVAWYQQKPGQAPRALIYSASLRFSGIPARFSGSGSGTEFTLTISSLQSEDFAVYYCQQYNNYPLTFGAGTKLELKR

SEQ ID NO: 50 - protein, 108 aa, synthetic construct
  REGION 1..108: note = VL
  REGION 30..31: note = misc_feature - Xaa can be any naturally occurring amino acid
EIVMTQSPATLSVSPGERATLSCKASQSVXXNVAWYQQKPGQAPRALIYSASLRFSGIPARFSGSGSGTEFTLTISSLQSEDFAVYYCQQYNNYPLTFGAGTKLELKR

SEQ ID NO: 51 - protein, 108 aa, synthetic construct
  REGION 1..108: note = VL
  REGION 31..32: note = misc_feature - Xaa can be any naturally occurring amino acid
  SITE 34: note = misc_feature - Xaa can be any naturally occurring amino acid
  SITE 36: note = misc_feature - Xaa can be any naturally occurring amino acid
  REGION 49..50: note = misc_feature - Xaa can be any naturally occurring amino acid
  REGION 52..53: note = misc_feature - Xaa can be any naturally occurring amino acid
  SITE 55: note = misc_feature - Xaa can be any naturally occurring amino acid
  REGION 66..67: note = misc_feature - Xaa can be any naturally occurring amino acid
  SITE 89: note = misc_feature - Xaa can be any naturally occurring amino acid
  SITE 91: note = misc_feature - Xaa can be any naturally occurring amino acid
  SITE 94: note = misc_feature - Xaa can be any naturally occurring amino acid
  SITE 96: note = misc_feature - Xaa can be any naturally occurring amino acid
EIVMTQSPATLSVSPGERATLSCKASQSVDXXVXWXQQKPGQAPRALIXXAXXRXSGIPARFSGSXXGTEFTLTISSLQSEDFAVYYCXQXNNXPXTFGAGTKLELKR

SEQ ID NO: 52 - protein, 108 aa, synthetic construct
  REGION 1..108: note = VL
EIVMTQSPATLSVSPGERATLSCKASQSVESNVAWYQQKPGQAPRALIYSASLRFSGIPARFSGSGSGTEFTLTISSLQSEDFAVYYCQQYNNYPLTFGAGTKLELKR

SEQ ID NO: 53 - protein, 120 aa, synthetic construct
  REGION 1..120: note = VH
  SITE 1: note = misc_feature - Xaa can be any naturally occurring amino acid
  REGION 5..6: note = misc_feature - Xaa can be any naturally occurring amino acid
  SITE 19: note = misc_feature - Xaa can be any naturally occurring amino acid
  REGION 27..28: note = misc_feature - Xaa can be any naturally occurring amino acid
  REGION 30..31: note = misc_feature - Xaa can be any naturally occurring amino acid
  SITE 34: note = misc_feature - Xaa can be any naturally occurring amino acid
  SITE 39: note = misc_feature - Xaa can be any naturally occurring amino acid
  SITE 48: note = misc_feature - Xaa can be any naturally occurring amino acid
  SITE 54: note = misc_feature - Xaa can be any naturally occurring amino acid
  REGION 66..67: note = misc_feature - Xaa can be any naturally occurring amino acid
  SITE 69: note = misc_feature - Xaa can be any naturally occurring amino acid
  REGION 84..86: note = misc_feature - Xaa can be any naturally occurring amino acid
  SITE 88: note = misc_feature - Xaa can be any naturally occurring amino acid
  SITE 93: note = misc_feature - Xaa can be any naturally occurring amino acid
  SITE 107: note = misc_feature - Xaa can be any naturally occurring amino acid
  SITE 115: note = misc_feature - Xaa can be any naturally occurring amino acid
XVQLXXSGGGLVQPGGSLXLSCAASGXXFXXYWXSWVRXAPGKGLEWXGEINPXSSTINYAPSLKXXFXISRDNAKNTLYLQMXXXRXEDTAXYYCASLYYDYGDAXDYWGQGTXVTVSS

SEQ ID NO: 54 - protein, 108 aa, synthetic construct
  REGION 1..108: note = VL
  REGION 8..13: note = misc_feature - Xaa can be any naturally occurring amino acid
  SITE 18: note = misc_feature - Xaa can be any naturally occurring amino acid
  REGION 20..21: note = misc_feature - Xaa can be any naturally occurring amino acid
  SITE 41: note = misc_feature - Xaa can be any naturally occurring amino acid
  SITE 43: note = misc_feature - Xaa can be any naturally occurring amino acid
  SITE 46: note = misc_feature - Xaa can be any naturally occurring amino acid
  SITE 49: note = misc_feature - Xaa can be any naturally occurring amino acid
  REGION 51..52: note = misc_feature - Xaa can be any naturally occurring amino acid
  SITE 63: note = misc_feature - Xaa can be any naturally occurring amino acid
  SITE 77: note = misc_feature - Xaa can be any naturally occurring amino acid
  SITE 83: note = misc_feature - Xaa can be any naturally occurring amino acid
  SITE 85: note = misc_feature - Xaa can be any naturally occurring amino acid
  SITE 87: note = misc_feature - Xaa can be any naturally occurring amino acid
DIVMTQSXXXXXXSVGDXVXXTCKASQSVESNVAWYQQKPXQXPKXLIXSXXLRFSGVPARFXGSGSGTDFTLTISXLQSEDXAXYXCQQYNNYPLTFGAGTKLELKR

SEQ ID NO: 55 - protein, 21 aa, synthetic construct
  REGION 1..21: note = leader
MDFQVQIFSFLLISASVIMSR

SEQ ID NO: 56 - protein, 21 aa, synthetic construct
  REGION 1..21: note = leader
MLLLVTSLLLCELPHPAFLLI

SEQ ID NO: 57 - protein, 684 aa, synthetic construct
  REGION 1..684: note = construct
MDFQVQIFSFLLISASVIMSREVQLVESGGGLVQPGGSLRLSCAASGFTFSRYWFSWVRQAPGKGLVWVGEINPSSSTINYAPSLKDKFTISRDNAKNTLYLQMNSLRAEDTAVYYCASLYYDYGDAYDYWGQGTLVTVSSGSTSGSGKPGSGEGSTKGEIVMTQSPATLSVSPGERATLSCKASQSVESNVAWYQQKPGQAPRALIYSASLRFSGIPARFSGSGSGTEFTLTISSLQSEDFAVYYCQQYNNYPLTFGAGTKLELKPAEPKSPDKTHTCPPCPAPPVAGPSVFLFPPKPKDTLMIARTPEVTCVVVDVSHEDPEVKFNWYVDGVEVHNAKTKPREEQYNSTYRVVSVLTVLHQDWLNGKEYKCKVSNKALPAPIEKTISKAKGQPREPQVYTLPPSRDELTKNQVSLTCLVKGFYPSDIAVEWESNGQPENNYKTTPPVLDSDGSFFLYSKLTVDKSRWQQGNVFSCSVMHEALHNHYTQKSLSLSPGKKDPKFWVLVVVGGVLACYSLLVTVAFIIFWVRSKRSRLLHSDYMNMTPRRPGPTRKHYQPYAPPRDFAAYRSLRVKFSRSADAPAYQQGQNQLYNELNLGRREEYDVLDKRRGRDPEMGGKPRRKNPQEGLYNELQKDKMAEAYSEIGMKGERRRGKGHDGLYQGLSTATKDTYDALHMQALPPR

SEQ ID NO: 58 - protein, 684 aa, synthetic construct
  REGION 1..684: note = construct
MDFQVQIFSFLLISASVIMSREIVMTQSPATLSVSPGERATLSCKASQSVESNVAWYQQKPGQAPRALIYSASLRFSGIPARFSGSGSGTEFTLTISSLQSEDFAVYYCQQYNNYPLTFGAGTKLELKGSTSGSGKPGSGEGSTKGEVQLVESGGGLVQPGGSLRLSCAASGFTFSRYWFSWVRQAPGKGLVWVGEINPSSSTINYAPSLKDKFTISRDNAKNTLYLQMNSLRAEDTAVYYCASLYYDYGDAYDYWGQGTLVTVSSPAEPKSPDKTHTCPPCPAPPVAGPSVFLFPPKPKDTLMIARTPEVTCVVVDVSHEDPEVKFNWYVDGVEVHNAKTKPREEQYNSTYRVVSVLTVLHQDWLNGKEYKCKVSNKALPAPIEKTISKAKGQPREPQVYTLPPSRDELTKNQVSLTCLVKGFYPSDIAVEWESNGQPENNYKTTPPVLDSDGSFFLYSKLTVDKSRWQQGNVFSCSVMHEALHNHYTQKSLSLSPGKKDPKFWVLVVVGGVLACYSLLVTVAFIIFWVRSKRSRLLHSDYMNMTPRRPGPTRKHYQPYAPPRDFAAYRSLRVKFSRSADAPAYQQGQNQLYNELNLGRREEYDVLDKRRGRDPEMGGKPRRKNPQEGLYNELQKDKMAEAYSEIGMKGERRRGKGHDGLYQGLSTATKDTYDALHMQALPPR

SEQ ID NO: 59 - protein, 684 aa, synthetic construct; identical to SEQ ID NO: 57
  REGION 1..684: note = construct

SEQ ID NO: 60 - protein, 676 aa, synthetic construct
  REGION 1..676: note = construct
MDFQVQIFSFLLISASVIMSREVQLVESGGGLVQPGGSLRLSCAASGFTFSRYWFSWVRQAPGKGLVWVGEINPSSSTINYAPSLKDKFTISRDNAKNTLYLQMNSLRAEDTAVYYCASLYYDYGDAYDYWGQGTLVTVSSGSTSGSGKPGSGEGSTKGEIVMTQSPATLSVSPGERATLSCKASQSVESNVAWYQQKPGQAPRALIYSASLRFSGIPARFSGSGSGTEFTLTISSLQSEDFAVYYCQQYNNYPLTFGAGTKLELKESKYGPPCPPCPAPEFEGGPSVFLFPPKPKDTLMISRTPEVTCVVVDVSQEDPEVQFNWYVDGVEVHNAKTKPREEQFNSTYRVVSVLTVLHQDWLNGKEYKCKVSNKGLPSSIEKTISKAKGQPREPQVYTLPPSQEEMTKNQVSLTCLVKGFYPSDIAVEWESNGQPENNYKTTPPVLDSDGSFFLYSRLTVDKSRWQEGNVFSCSVMHEALHNHYTQKSLSLSLGKFWVLVVVGGVLACYSLLVTVAFIIFWVRSKRSRLLHSDYMNMTPRRPGPTRKHYQPYAPPRDFAAYRSLRVKFSRSADAPAYQQGQNQLYNELNLGRREEYDVLDKRRGRDPEMGGKPRRKNPQEGLYNELQKDKMAEAYSEIGMKGERRRGKGHDGLYQGLSTATKDTYDALHMQALPPR

SEQ ID NO: 61 - protein, 566 aa, synthetic construct
  REGION 1..566: note = construct
MDFQVQIFSFLLISASVIMSREVQLVESGGGLVQPGGSLRLSCAASGFTFSRYWFSWVRQAPGKGLVWVGEINPSSSTINYAPSLKDKFTISRDNAKNTLYLQMNSLRAEDTAVYYCASLYYDYGDAYDYWGQGTLVTVSSGSTSGSGKPGSGEGSTKGEIVMTQSPATLSVSPGERATLSCKASQSVESNVAWYQQKPGQAPRALIYSASLRFSGIPARFSGSGSGTEFTLTISSLQSEDFAVYYCQQYNNYPLTFGAGTKLELKESKYGPPCPPCPGQPREPQVYTLPPSQEEMTKNQVSLTCLVKGFYPSDIAVEWESNGQPENNYKTTPPVLDSDGSFFLYSRLTVDKSRWQEGNVFSCSVMHEALHNHYTQKSLSLSLGKFWVLVVVGGVLACYSLLVTVAFIIFWVRSKRSRLLHSDYMNMTPRRPGPTRKHYQPYAPPRDFAAYRSLRVKFSRSADAPAYQQGQNQLYNELNLGRREEYDVLDKRRGRDPEMGGKPRRKNPQEGLYNELQKDKMAEAYSEIGMKGERRRGKGHDGLYQGLSTATKDTYDALHMQALPPR

SEQ ID NO: 62 - protein, 459 aa, synthetic construct
  REGION 1..459: note = construct
MDFQVQIFSFLLISASVIMSREVQLVESGGGLVQPGGSLRLSCAASGFTFSRYWFSWVRQAPGKGLVWVGEINPSSSTINYAPSLKDKFTISRDNAKNTLYLQMNSLRAEDTAVYYCASLYYDYGDAYDYWGQGTLVTVSSGSTSGSGKPGSGEGSTKGEIVMTQSPATLSVSPGERATLSCKASQSVESNVAWYQQKPGQAPRALIYSASLRFSGIPARFSGSGSGTEFTLTISSLQSEDFAVYYCQQYNNYPLTFGAGTKLELKESKYGPPCPPCPFWVLVVVGGVLACYSLLVTVAFIIFWVRSKRSRLLHSDYMNMTPRRPGPTRKHYQPYAPPRDFAAYRSLRVKFSRSADAPAYQQGQNQLYNELNLGRREEYDVLDKRRGRDPEMGGKPRRKNPQEGLYNELQKDKMAEAYSEIGMKGERRRGKGHDGLYQGLSTATKDTYDALHMQALPPR

SEQ ID NO: 63 - protein, 680 aa, synthetic construct
  REGION 1..680: note = construct
MDFQVQIFSFLLISASVIMSREVQLVESGGGLVQPGGSLRLSCAASGFTFSRYWFSWVRQAPGKGLVWVGEINPSSSTINYAPSLKDKFTISRDNAKNTLYLQMNSLRAEDTAVYYCASLYYDYGDAYDYWGQGTLVTVSSGSTSGSGKPGSGEGSTKGEIVMTQSPATLSVSPGERATLSCKASQSVESNVAWYQQKPGQAPRALIYSASLRFSGIPARFSGSGSGTEFTLTISSLQSEDFAVYYCQQYNNYPLTFGAGTKLELKPAEPKSPDKTHTCPPCPAPPVAGPSVFLFPPKPKDTLMIARTPEVTCVVVDVSHEDPEVKFNWYVDGVEVHNAKTKPREEQYNSTYRVVSVLTVLHQDWLNGKEYKCKVSNKALPAPIEKTISKAKGQPREPQVYTLPPSRDELTKNQVSLTCLVKGFYPSDIAVEWESNGQPENNYKTTPPVLDSDGSFFLYSKLTVDKSRWQQGNVFSCSVMHEALHNHYTQKSLSSLSPGKKIYIWAPLAGTCGVLLLSLVITLYCKRGRKKLLYIFKQPFMRPVQTTQEEDGCSCRFPEEEEGGCELLRVKFSRSADAPAYQQGQNQLYNELNLGRREEYDVLDKRRGRDPEMGGKPRRKNPQEGLYNELQKDKMAEAYSEIGMKGERRRGKGHDGLYQGLSTATKDTYDALHMQALPPR

SEQ ID NO: 64 - protein, 680 aa, synthetic construct
  REGION 1..680: note = construct
MDFQVQIFSFLLISASVIMSREIVMTQSPATLSVSPGERATLSCKASQSVESNVAWYQQKPGQAPRALIYSASLRFSGIPARFSGSGSGTEFTLTISSLQSEDFAVYYCQQYNNYPLTFGAGTKLELKGSTSGSGKPGSGEGSTKGEVQLVESGGGLVQPGGSLRLSCAASGFTFSRYWFSWVRQAPGKGLVWVGEINPSSSTINYAPSLKDKFTISRDNAKNTLYLQMNSLRAEDTAVYYCASLYYDYGDAYDYWGQGTLVTVSSPAEPKSPDKTHTCPPCPAPPVAGPSVFLFPPKPKDTLMIARTPEVTCVVVDVSHEDPEVKFNWYVDGVEVHNAKTKPREEQYNSTYRVVSVLTVLHQDWLNGKEYKCKVSNKALPAPIEKTISKAKGQPREPQVYTLPPSRDELTKNQVSLTCLVKGFYPSDIAVEWESNGQPENNYKTTPPVLDSDGSFFLYSKLTVDKSRWQQGNVFSCSVMHEALHNHYTQKSLSSLSPGKKIYIWAPLAGTCGVLLLSLVITLYCKRGRKKLLYIFKQPFMRPVQTTQEEDGCSCRFPEEEEGGCELLRVKFSRSADAPAYQQGQNQLYNELNLGRREEYDVLDKRRGRDPEMGGKPRRKNPQEGLYNELQKDKMAEAYSEIGMKGERRRGKGHDGLYQGLSTATKDTYDALHMQALPPR

SEQ ID NO: 65 - protein, 680 aa, synthetic construct; identical to SEQ ID NO: 63
  REGION 1..680: note = construct

SEQ ID NO: 66 - DNA, 360 bp, synthetic construct
  misc_feature 1..360: note = VH
  source 1..360: mol_type = other DNA
gaggtgcagctggtggaatctggcggaggactggtgcagcctggcggctctctgagactgtcttgtgccgccagcggcttcaccttcagccggtactggtttagctgggtgcgccaggcccctggcaagggactcgtgtgggtgggagagatcaaccccagcagcagcaccatcaactacgcccccagcctgaaggacaagttcaccatcagcagagacaacgccaagaacaccctgtacctgcagatgaacagcctgcgggccgaggacaccgccgtgtactattgtgccagcctgtactacgactacggcgacgcctacgattactggggccagggcacactggtgactgttagctcc

SEQ ID NO: 67 - DNA, 321 bp, synthetic construct
  misc_feature 1..321: note = VL
  source 1..321: mol_type = other DNA
gagatcgtgatgacacagagccctgccaccctgagcgtgtccccaggcgaaagagctaccctgagctgcaaggccagccagagcgtggaaagcaacgtggcctggtatcagcagaagcccggacaggctcctcgggccctgatctacagcgccagcctgagattcagcggcatccccgccaggtttagcggctctggcagcggcaccgagttcaccctgacaatcagcagcctgcagagcgaggactttgccgtgtattactgccagcagtacaacaactaccccctgaccttcggagccggcaccaagctggagctgaag

SEQ ID NO: 68 - DNA, 360 bp, synthetic construct
  misc_feature 1..360: note = VH
  source 1..360: mol_type = other DNA
gaagtgcagctggtcgaatctggaggaggcctggttcagcctggtggcagccttaggctctcttgtgcagcctctggctttaccttctcacggtattggttcagctgggtgagacaggctccagggaaaggtctggtgtgggtaggggagataaaccccagcagcagcacgatcaactatgctccgtcactgaaagacaagttcaccatttcccgcgataatgccaagaacactctctacttgcagatgaattcccttcgagccgaggatacagcggtgtactactgcgccagtctgtactacgactatggggacgcatacgactattggggacaaggcacactggtgactgttagctcc

SEQ ID NO: 69 - DNA, 321 bp, synthetic construct
  misc_feature 1..321: note = VL
  source 1..321: mol_type = other DNA
gagatcgtgatgacccagtctcctgctaccctgagcgtttctcccggtgaaagggccacactcagctgcaaagcctctcaaagcgtggagagcaatgtcgcctggtatcagcagaaacctggccaagctccgagagcactgatctattccgcgtcattgcgcttttccggcataccagcacggtttagtggctcagggagtgggactgagttcactctgacgattagctcccttcagtcagaggatttcgccgtgtactactgtcagcagtacaacaactatcccctcacattcggagctggaaccaagctggaactgaag

SEQ ID NO: 70 - DNA, 63 bp, synthetic construct
  misc_feature 1..63: note = leader
  source 1..63: mol_type = other DNA
atggatttccaggtgcagatcttcagcttcctgctgatctccgccagcgtgatcatgagccgc

SEQ ID NO: 71 - DNA, 63 bp, synthetic construct
  misc_feature 1..63: note = leader
  source 1..63: mol_type = other DNA
atgcttctcctggtgacaagccttctgctctgtgagttaccacacccagcattcctcctgatc

SEQ ID NO: 72 - DNA, 54 bp, synthetic construct
  misc_feature 1..54: note = linker
  source 1..54: mol_type = other DNA
ggcagcaccagcggctccggcaagcctggctctggcgagggcagcacaaaggga

SEQ ID NO: 73 - DNA, 51 bp, synthetic construct
  misc_feature 1..51: note = linker
  source 1..51: mol_type = other DNA
tctagcggcggaggcggatctggcgggggaggatctgggggaggcggctct

SEQ ID NO: 74 - DNA, 702 bp, synthetic construct
  misc_feature 1..702: note = spacer
  source 1..702: mol_type = other DNA
cctgccgagcctaagagccccgacaagacccacacctgtcccccttgtcctgcccctccagtggctggccctagcgtgttcctgttccccccaaagcccaaggataccctgatgatcgcccggacccccgaagtcacatgcgtggtggtggacgtgagccacgaagaccctgaggtcaagttcaactggtacgtggacggcgtggaggtgcataatgccaagacaaagccgcgggaggagcagtacaacagcacgtaccgtgtggtcagcgtcctcaccgtcctgcaccaggactggctgaatggcaaggagtacaagtgcaaggtctccaacaaagccctcccagcccccatcgagaaaaccatctccaaagccaaagggcagccccgagaaccacaggtgtacaccctgcccccatcccgggatgagctgaccaagaaccaggtcagcctgacctgcctggtcaaaggcttctatcccagcgacatcgccgtggagtgggagagcaatgggcagccggagaacaactacaagaccacgcctcccgtgctggactccgacggctccttcttcctctacagcaagctcaccgtggacaagagcaggtggcagcaggggaacgtcttctcatgctccgtgatgcatgaggctctgcacaaccactacacgcagaagagcctctccctgtctccgggtaaaaaa

SEQ ID NO: 75 - DNA, 705 bp, synthetic construct
  misc_feature 1..705: note = spacer
  source 1..705: mol_type = other DNA
cctgccgagcctaagagccccgacaagacccacacctgtcccccttgtcctgcccctccagtggctggccctagcgtgttcctgttccccccaaagcccaaggataccctgatgatcgcccggacccccgaagtcacatgcgtggtggtggacgtgagccacgaagaccctgaggtcaagttcaactggtacgtggacggcgtggaggtgcataatgccaagacaaagccgcgggaggagcagtacaacagcacgtaccgtgtggtcagcgtcctcaccgtcctgcaccaggactggctgaatggcaaggagtacaagtgcaaggtctccaacaaagccctcccagcccccatcgagaaaaccatctccaaagccaaagggcagccccgagaaccacaggtgtacaccctgcccccatcccgggatgagctgaccaagaaccaggtgtccctgacctgcctcgtgaagggcttctacccctccgatatcgccgtggaatgggagagcaatggccagcccgagaacaactacaagaccaccccccctgtgctggacagcgacggctcattcttcctgtacagcaagctgacagtggacaagagccggtggcagcagggcaacgtgttcagctgcagcgtgatgcacgaggctctgcacaaccactacacccagaagtccctgagcagcctgagcccaggcaagaag

SEQ ID NO: 76 - DNA, 687 bp, synthetic construct
  misc_feature 1..687: note = spacer
  source 1..687: mol_type = other DNA
gagagcaagtacggccctccctgccccccttgccctgcccccgagttcgagggcggacccagcgtgttcctgttcccccccaagcccaaggacaccctgatgatcagccggacccccgaggtgacctgcgtggtggtggacgtgagccaggaagatcccgaggtccagttcaattggtacgtggacggcgtggaagtgcacaacgccaagaccaagcccagagaggaacagttcaacagcacctaccgggtggtgtctgtgctgaccgtgctgcaccaggactggctgaacggcaaagaatacaagtgcaaggtgtccaacaagggcctgcccagcagcatcgaaaagaccatcagcaaggccaagggccagcctcgcgagccccaggtgtacaccctgcctccctcccaggaagagatgaccaagaaccaggtgtccctgacctgcctggtgaagggcttctaccccagcgacatcgccgtggagtgggagagcaacggccagcctgagaacaactacaagaccacccctcccgtgctggacagcgacggcagcttcttcctctacagccggctgaccgtggacaagagccggtggcaggaaggcaacgtctttagctgcagcgtgatgcacgaggccctgcacaaccactacacccagaagagcctgagcctgtccctgggcaag

SEQ ID NO: 77 - DNA, 357 bp, synthetic construct
  misc_feature 1..357: note = spacer
  source 1..357: mol_type = other DNA
gagagcaagtacggccctccctgccccccttgccctggccagcctcgcgagccccaggtgtacaccctgcctccctcccaggaagagatgaccaagaaccaggtgtccctgacctgcctggtgaagggcttctaccccagcgacatcgccgtggagtgggagagcaacggccagcctgagaacaactacaagaccacccctcccgtgctggacagcgacggcagcttcttcctctacagccggctgaccgtggacaagagccggtggcaggaaggcaacgtctttagctgcagcgtgatgcacgaggccctgcacaaccactacacccagaagagcctgagcctgtccctgggcaag

SEQ ID NO: 78 - DNA, 36 bp, synthetic construct
  misc_feature 1..36: note = spacer
  source 1..36: mol_type = other DNA
gagagcaagtacggccctccctgccccccttgccct

SEQ ID NO: 79 - DNA, 72 bp, synthetic construct
  misc_feature 1..72: note = transmembrane
  source 1..72: mol_type = other DNA
atctacatctgggcccctctggccggcacctgtggcgtgctgctgctgtctctcgtgatcacactgtactgc

SEQ ID NO: 80 - DNA, 81 bp, synthetic construct
  misc_feature 1..81: note = transmembrane
  source 1..81: mol_type = other DNA
ttttgggtgctggtggtggttggtggagtcctggcttgctatagcttgctagtaacagtggcctttattattttctgggtg

SEQ ID NO: 81 - DNA, 126 bp, synthetic construct
  misc_feature 1..126: note = intracellular
  source 1..126: mol_type = other DNA
aagcggggcagaaagaagctgctgtacatcttcaagcagcccttcatgcggcccgtgcagaccacccaggaagaggacggctgctcctgcagattccccgaggaagaagaaggcggctgcgagctg

SEQ ID NO: 82 - DNA, 123 bp, synthetic construct
  misc_feature 1..123: note = intracellular
  source 1..123: mol_type = other DNA
aggagtaagaggagcaggctcctgcacagtgactacatgaacatgactccccgccgccccgggcccacccgcaagcattaccagccctatgccccaccacgcgacttcgcagcctatcgctcc

SEQ ID NO: 83 - DNA, 123 bp, synthetic construct
  misc_feature 1..123: note = intracellular
  source 1..123: mol_type = other DNA
aggagtaagaggagcaggctcctgcacagtgactacatgaacatgactccccgtcgacccgggcccacccgcaagcattaccagccctatgccccaccacgcgacttcgcagcctatcgctcc

SEQ ID NO: 84 - DNA, 342 bp, synthetic construct
  misc_feature 1..342: note = intracellular
  source 1..342: mol_type = other DNA
ctgagagtgaagttcagcaggagcgcagacgcccccgcgtaccagcagggccagaaccagctctataacgagctcaatctaggacgaagagaggagtacgatgttttggacaagagacgtggccgggaccctgagatggggggaaagccgagaaggaagaaccctcaggaaggcctgtacaatgaactgcagaaagataagatggcggaggcctacagtgagattgggatgaaaggcgagcgccggaggggcaaggggcacgatggcctttaccagggtctcagtacagccaccaaggacacctacgacgcccttcacatgcaggccctgccccctcgctga

SEQ ID NO: 85 - DNA, 339 bp, synthetic construct
  misc_feature 1..339: note = intracellular
  source 1..339: mol_type = other DNA
ctgcgcgtgaagttttctagaagcgccgacgcccctgcctaccagcagggccagaaccagctgtacaacgagctgaacctgggcagacgggaagagtacgacgtgctggataagcggagaggccgggaccctgagatgggcggcaagcctagaagaaagaacccccaggaaggcctgtataacgaactgcagaaagacaagatggccgaggcctacagcgagatcggaatgaagggcgagcggagaagaggcaagggccacgatggactgtaccagggcctgagcaccgccaccaaggacacctatgacgccctgcacatgcaggctctgccccccaga

SEQ ID NO: 86 - DNA, 2055 bp, synthetic construct
  misc_feature 1..2055: note = construct
  source 1..2055: mol_type = other DNA
atggatttccaggtgcagatcttcagcttcctgctgatctccgccagcgtgatcatgagccgcgaggtgcagctggtggaatctggcggaggactggtgcagcctggcggctctctgagactgtcttgtgccgccagcggcttcaccttcagccggtactggtttagctgggtgcgccaggcccctggcaagggactcgtgtgggtgggagagatcaaccccagcagcagcaccatcaactacgcccccagcctgaaggacaagttcaccatcagcagagacaacgccaagaacaccctgtacctgcagatgaacagcctgcgggccgaggacaccgccgtgtactattgtgccagcctgtactacgactacggcgacgcctacgattactggggccagggcacactggtgactgttagctccggcagcaccagcggctccggcaagcctggctctggcgagggcagcacaaagggagagatcgtgatgacacagagccctgccaccctgagcgtgtccccaggcgaaagagctaccctgagctgcaaggccagccagagcgtggaaagcaacgtggcctggtatcagcagaagcccggacaggctcctcgggccctgatctacagcgccagcctgagattcagcggcatccccgccaggtttagcggctctggcagcggcaccgagttcaccctgacaatcagcagcctgcagagcgaggactttgccgtgtattactgccagcagtacaacaactaccccctgaccttcggagccggcaccaagctggagctgaagcctgccgagcctaagagccccgacaagacccacacctgtcccccttgtcctgcccctccagtggctggccctagcgtgttcctgttccccccaaagcccaaggataccctgatgatcgcccggacccccgaagtcacatgcgtggtggtggacgtgagccacgaagaccctgaggtcaagttcaactggtacgtggacggcgtggaggtgcataatgccaagacaaagccgcgggaggagcagtacaacagcacgtaccgtgtggtcagcgtcctcaccgtcctgcaccaggactggctgaatggcaaggagtacaagtgcaaggtctccaacaaagccctcccagcccccatcgagaaaaccatctccaaagccaaagggcagccccgagaaccacaggtgtacaccctgcccccatcccgggatgagctgaccaagaaccaggtcagcctgacctgcctggtcaaaggcttctatcccagcgacatcgccgtggagtgggagagcaatgggcagccggagaacaactacaagaccacgcctcccgtgctggactccgacggctccttcttcctctacagcaagctcaccgtggacaagagcaggtggcagcaggggaacgtcttctcatgctccgtgatgcatgaggctctgcacaaccactacacgcagaagagcctctccctgtctccgggtaaaaaagatcccaaattttgggtgctggtggtggttggtggagtcctggcttgctatagcttgctagtaacagtggcctttattattttctgggtgaggagtaagaggagcaggctcctgcacagtgactacatgaacatgactccccgccgccccgggcccacccgcaagcattaccagccctatgccccaccacgcgacttcgcagcctatcgctccctgagagtgaagttcagcaggagcgcagacgcccccgcgtaccagcagggccagaaccagctctataacgagctcaatctaggacgaagagaggagtacgatgttttggacaagagacgtggccgggaccctgagatggggggaaagccgagaaggaagaaccctcaggaaggcctgtacaatgaactgcagaaagataagatggcggaggcctacagtgagattgggatgaaaggcgagcgccggaggggcaaggggcacgatggcctttaccagggtctcagtacagccaccaaggacacctacgacgcccttcacatgcaggccctgccccctcgctga

SEQ ID NO: 87 - DNA, 2055 bp, synthetic construct
  misc_feature 1..2055: note = construct
  source 1..2055: mol_type = other DNA
atggatttccaggtgcagatcttcagcttcctgctgatctccgccagcgtgatcatgagccgcgagatcgtgatgacacagagccctgccaccctgagcgtgtccccaggcgaaagagctaccctgagctgcaaggccagccagagcgtggaaagcaacgtggcctggtatcagcagaagcccggacaggctcctcgggccctgatctacagcgccagcctgagattcagcggcatccccgccaggtttagcggctctggcagcggcaccgagttcaccctgacaatcagcagcctgcagagcgaggactttgccgtgtattactgccagcagtacaacaactaccccctgaccttcggagccggcaccaagctggagctgaagggcagcaccagcggctccggcaagcctggctctggcgagggcagcacaaagggagaggtgcagctggtggaatctggcggaggactggtgcagcctggcggctctctgagactgtcttgtgccgccagcggcttcaccttcagccggtactggtttagctgggtgcgccaggcccctggcaagggactcgtgtgggtgggagagatcaaccccagcagcagcaccatcaactacgcccccagcctgaaggacaagttcaccatcagcagagacaacgccaagaacaccctgtacctgcagatgaacagcctgcgggccgaggacaccgccgtgtactattgtgccagcctgtactacgactacggcgacgcctacgattactggggccagggcacactggtgactgttagctcccctgccgagcctaagagccccgacaagacccacacctgtcccccttgtcctgcccctccagtggctggccctagcgtgttcctgttccccccaaagcccaaggataccctgatgatcgcccggacccccgaagtcacatgcgtggtggtggacgtgagccacgaagaccctgaggtcaagttcaactggtacgtggacggcgtggaggtgcataatgccaagacaaagccgcgggaggagcagtacaacagcacgtaccgtgtggtcagcgtcctcaccgtcctgcaccaggactggctgaatggcaaggagtacaagtgcaaggtctccaacaaagccctcccagcccccatcgagaaaaccatctccaaagccaaagggcagccccgagaaccacaggtgtacaccctgcccccatcccgggatgagctgaccaagaaccaggtcagcctgacctgcctggtcaaaggcttctatcccagcgacatcgccgtggagtgggagagcaatgggcagccggagaacaactacaagaccacgcctcccgtgctggactccgacggctccttcttcctctacagcaagctcaccgtggacaagagcaggtggcagcaggggaacgtcttctcatgctccgtgatgcatgaggctctgcacaaccactacacgcagaagagcctctccctgtctccgggtaaaaaagatcccaaattttgggtgctggtggtggttggtggagtcctggcttgctatagcttgctagtaacagtggcctttattattttctgggtgaggagtaagaggagcaggctcctgcacagtgactacatgaacatgactccccgccgccccgggcccacccgcaagcattaccagccctatgccccaccacgcgacttcgcagcctatcgctccctgagagtgaagttcagcaggagcgcagacgcccccgcgtaccagcagggccagaaccagctctataacgagctcaatctaggacgaagagaggagtacgatgttttggacaagagacgtggccgggaccctgagatggggggaaagccgagaaggaagaaccctcaggaaggcctgtacaatgaactgcagaaagataagatggcggaggcctacagtgagattgggatgaaaggcgagcgccggaggggcaaggggcacgatggcctttaccagggtctcagtacagccaccaaggacacctacgacgcccttcacatgcaggccctgccccctcgctga

SEQ ID NO: 88 - DNA, 2055 bp, synthetic construct
  misc_feature 1..2055: note = construct
  source 1..2055: mol_type = other DNA
atggatttccaggtgcagatcttcagcttcctgctgatctccgccagcgtgatcatgagccgcgaagtgcagctggtcgaatctggaggaggcctggttcagcctggtggcagccttaggctctcttgtgcagcctctggctttaccttctcacggtattggttcagctgggtgagacaggctccagggaaaggtctggtgtgggtaggggagataaaccccagcagcagcacgatcaactatgctccgtcactgaaagacaagttcaccatttcccgcgataatgccaagaacactctctacttgcagatgaattcccttcgagccgaggatacagcggtgtactactgcgccagtctgtactacgactatggggacgcatacgactattggggacaaggcacactggtgactgttagctccggcagcaccagcggctccggcaagcctggctctggcgagggcagcacaaagggagagatcgtgatgacccagtctcctgctaccctgagcgtttctcccggtgaaagggccacactcagctgcaaagcctctcaaagcgtggagagcaatgtcgcctggtatcagcagaaacctggccaagctccgagagcactgatctattccgcgtcattgcgcttttccggcataccagcacggtttagtggctcagggagtgggactgagttcactctgacgattagctcccttcagtcagaggatttcgccgtgtactactgtcagcagtacaacaactatcccctcacattcggagctggaaccaagctggaactgaagcctgccgagcctaagagccccgacaagacccacacctgtcccccttgtcctgcccctccagtggctggccctagcgtgttcctgttccccccaaagcccaaggataccctgatgatcgcccggacccccgaagtcacatgcgtggtggtggacgtgagccacgaagaccctgaggtcaagttcaactggtacgtggacggcgtggaggtgcataatgccaagacaaagccgcgggaggagcagtacaacagcacgtaccgtgtggtcagcgtcctcaccgtcctgcaccaggactggctgaatggcaaggagtacaagtgcaaggtctccaacaaagccctcccagcccccatcgagaaaaccatctccaaagccaaagggcagccccgagaaccacaggtgtacaccctgcccccatcccgggatgagctgaccaagaaccaggtcagcctgacctgcctggtcaaaggcttctatcccagcgacatcgccgtggagtgggagagcaatgggcagccggagaacaactacaagaccacgcctcccgtgctggactccgacggctccttcttcctctacagcaagctcaccgtggacaagagcaggtggcagcaggggaacgtcttctcatgctccgtgatgcatgaggctctgcacaaccactacacgcagaagagcctctccctgtctccgggtaaaaaagatcccaaattttgggtgctggtggtggttggtggagtcctggcttgctatagcttgctagtaacagtggcctttattattttctgggtgaggagtaagaggagcaggctcctgcacagtgactacatgaacatgactccccgccgccccgggcccacccgcaagcattaccagccctatgccccaccacgcgacttcgcagcctatcgctccctgagagtgaagttcagcaggagcgcagacgcccccgcgtaccagcagggccagaaccagctctataacgagctcaatctaggacgaagagaggagtacgatgttttggacaagagacgtggccgggaccctgagatggggggaaagccgagaaggaagaaccctcaggaaggcctgtacaatgaactgcagaaagataagatggcggaggcctacagtgagattgggatgaaaggcgagcgccggaggggcaaggggcacgatggcctttaccagggtctcagtacagccaccaaggacacctacgacgcccttcacatgcaggccctgccccctcgctga

SEQ ID NO: 89 - DNA, 2031 bp, synthetic construct
  misc_feature 1..2031: note = construct
  source 1..2031: mol_type = other DNA
atggatttccaggtgcagatcttcagcttcctgctgatctccgccagcgtgatcatgagccgcgaggtgcagctggtggaatctggcggaggactggtgcagcctggcggctctctgagactgtcttgtgccgccagcggcttcaccttcagccggtactggtttagctgggtgcgccaggcccctggcaagggactcgtgtgggtgggagagatcaaccccagcagcagcaccatcaactacgcccccagcctgaaggacaagttcaccatcagcagagacaacgccaagaacaccctgtacctgcagatgaacagcctgcgggccgaggacaccgccgtgtactattgtgccagcctgtactacgactacggcgacgcctacgattactggggccagggcacactggtgactgttagctccggcagcaccagcggctccggcaagcctggctctggcgagggcagcacaaagggagagatcgtgatgacacagagccctgccaccctgagcgtgtccccaggcgaaagagctaccctgagctgcaaggccagccagagcgtggaaagcaacgtggcctggtatcagcagaagcccggacaggctcctcgggccctgatctacagcgccagcctgagattcagcggcatccccgccaggttttccggatctggcagcggcaccgagttcaccctgacaatcagcagcctgcagagcgaggactttgccgtgtattactgccagcagtacaacaactaccccctgaccttcggagccggcaccaagctggagctgaaggagagcaagtacggccctccctgccccccttgccctgcccccgagttcgagggcggacccagcgtgttcctgttcccccccaagcccaaggacaccctgatgatcagccggacccccgaggtgacctgcgtggtggtggacgtgagccaggaagatcccgaggtccagttcaattggtacgtggacggcgtggaagtgcacaacgccaagaccaagcccagagaggaacagttcaacagcacctaccgggtggtgtctgtgctgaccgtgctgcaccaggactggctgaacggcaaagaatacaagtgcaaggtgtccaacaagggcctgcccagcagcatcgaaaagaccatcagcaaggccaagggccagcctcgcgagccccaggtgtacaccctgcctccctcccaggaagagatgaccaagaaccaggtgtccctgacctgcctggtgaagggcttctaccccagcgacatcgccgtggagtgggagagcaacggccagcctgagaacaactacaagaccacccctcccgtgctggacagcgacggcagcttcttcctctacagccggctgaccgtggacaagagccggtggcaggaaggcaacgtctttagctgcagcgtgatgcacgaggccctgcacaaccactacacccagaagagcctgagcctgtccctgggcaagttttgggtgctggtggtggttggtggagtcctggcttgctatagcttgctagtaacagtggcctttattattttctgggtgaggagtaagaggagcaggctcctgcacagtgactacatgaacatgactccccgtcgacccgggcccacccgcaagcattaccagccctatgccccaccacgcgacttcgcagcctatcgctccctgagagtgaagttcagcaggagcgcagacgcccccgcgtaccagcagggccagaaccagctctataacgagctcaatctaggacgaagagaggagtacgatgttttggacaagagacgtggccgggaccctgagatggggggaaagccgagaaggaagaaccctcaggaaggcctgtacaatgaactgcagaaagataagatggcggaggcctacagtgagattgggatgaaaggcgagcgccggaggggcaaggggcacgatggcctttaccagggtctcagtacagccaccaaggacacctacgacgcccttcacatgcaggccctgccccctcgctga

SEQ ID NO: 90 - DNA, 1701 bp, synthetic construct
  misc_feature 1..1701: note = construct
  source 1..1701: mol_type = other DNA
atggatttccaggtgcagatcttcagcttcctgctgatctccgccagcgtgatcatgagccgcgaggtgcagctggtggaatctggcggaggactggtgcagcctggcggctctctgagactgtcttgtgccgccagcggcttcaccttcagccggtactggtttagctgggtgcgccaggcccctggcaagggactcgtgtgggtgggagagatcaaccccagcagcagcaccatcaactacgcccccagcctgaaggacaagttcaccatcagcagagacaacgccaagaacaccctgtacctgcagatgaacagcctgcgggccgaggacaccgccgtgtactattgtgccagcctgtactacgactacggcgacgcctacgattactggggccagggcacactggtgactgttagctccggcagcaccagcggctccggcaagcctggctctggcgagggcagcacaaagggagagatcgtgatgacacagagccctgccaccctgagcgtgtccccaggcgaaagagctaccctgagctgcaaggccagccagagcgtggaaagcaacgtggcctggtatcagcagaagcccggacaggctcctcgggccctgatctacagcgccagcctgagattcagcggcatccccgccaggttttccggatctggcagcggcaccgagttcaccctgacaatcagcagcctgcagagcgaggactttgccgtgtattactgccagcagtacaacaactaccccctgaccttcggagccggcaccaagctggagctgaaggagagcaagtacggccctccctgccccccttgccctggccagcctcgcgagccccaggtgtacaccctgcctccctcccaggaagagatgaccaagaaccaggtgtccctgacctgcctggtgaagggcttctaccccagcgacatcgccgtggagtgggagagcaacggccagcctgagaacaactacaagaccacccctcccgtgctggacagcgacggcagcttcttcctctacagccggctgaccgtggacaagagccggtggcaggaaggcaacgtctttagctgcagcgtgatgcacgaggccctgcacaaccactacacccagaagagcctgagcctgtccctgggcaagttttgggtgctggtggtggttggtggagtcctggcttgctatagcttgctagtaacagtggcctttattattttctgggtgaggagtaagaggagcaggctcctgcacagtgactacatgaacatgactccccgtcgacccgggcccacccgcaagcattaccagccctatgccccaccacgcgacttcgcagcctatcgctccctgagagtgaagttcagcaggagcgcagacgcccccgcgtaccagcagggccagaaccagctctataacgagctcaatctaggacgaagagaggagtacgatgttttggacaagagacgtggccgggaccctgagatggggggaaagccgagaaggaagaaccctcaggaaggcctgtacaatgaactgcagaaagataagatggcggaggcctacagtgagattgggatgaaaggcgagcgccggaggggcaaggggcacgatggcctttaccagggtctcagtacagccaccaaggacacctacgacgcccttcacatgcaggccctgccccctcgctga

SEQ ID NO: 91 - DNA, 1380 bp, synthetic construct
  misc_feature 1..1380: note = construct
  source 1..1380: mol_type = other DNA
atggatttccaggtgcagatcttcagcttcctgctgatctccgccagcgtgatcatgagccgcgaggtgcagctggtggaatctggcggaggactggtgcagcctggcggctctctgagactgtcttgtgccgccagcggcttcaccttcagccggtactggtttagctgggtgcgccaggcccctggcaagggactcgtgtgggtgggagagatcaaccccagcagcagcaccatcaactacgcccccagcctgaaggacaagttcaccatcagcagagacaacgccaagaacaccctgtacctgcagatgaacagcctgcgggccgaggacaccgccgtgtactattgtgccagcctgtactacgactacggcgacgcctacgattactggggccagggcacactggtgactgttagctccggcagcaccagcggctccggcaagcctggctctggcgagggcagcacaaagggagagatcgtgatgacacagagccctgccaccctgagcgtgtccccaggcgaaagagctaccctgagctgcaaggccagccagagcgtggaaagcaacgtggcctggtatcagcagaagcccggacaggctcctcgggccctgatctacagcgccagcctgagattcagcggcatccccgccaggttttccggatctggcagcggcaccgagttcaccctgacaatcagcagcctgcagagcgaggactttgccgtgtattactgccagcagtacaacaactaccccctgaccttcggagccggcaccaagctggagctgaaggagagcaagtacggccctccctgccccccttgccctttttgggtgctggtggtggttggtggagtcctggcttgctatagcttgctagtaacagtggcctttattattttctgggtgaggagtaagaggagcaggctcctgcacagtgactacatgaacatgactccccgtcgacccgggcccacccgcaagcattaccagccctatgccccaccacgcgacttcgcagcctatcgctccctgagagtgaagttcagcaggagcgcagacgcccccgcgtaccagcagggccagaaccagctctataacgagctcaatctaggacgaagagaggagtacgatgttttggacaagagacgtggccgggaccctgagatggggggaaagccgagaaggaagaaccctcaggaaggcctgtacaatgaactgcagaaagataagatggcggaggcctacagtgagattgggatgaaaggcgagcgccggaggggcaaggggcacgatggcctttaccagggtctcagtacagccaccaaggacacctacgacgcccttcacatgcaggccctgccccctcgctga

SEQ ID NO: 92 - DNA, 2040 bp, synthetic construct
  misc_feature 1..2040: note = construct
  source 1..2040: mol_type = other DNA
atggatttccaggtgcagatcttcagcttcctgctgatctccgccagcgtgatcatgagccgcgaggtgcagctggtggaatctggcggaggactggtgcagcctggcggctctctgagactgtcttgtgccgccagcggcttcaccttcagccggtactggtttagctgggtgcgccaggcccctggcaagggactcgtgtgggtgggagagatcaaccccagcagcagcaccatcaactacgcccccagcctgaaggacaagttcaccatcagcagagacaacgccaagaacaccctgtacctgcagatgaacagcctgcgggccgaggacaccgccgtgtactattgtgccagcctgtactacgactacggcgacgcctacgattactggggccagggcacactggtgactgttagctccggcagcaccagcggctccggcaagcctggctctggcgagggcagcacaaagggagagatcgtgatgacacagagccctgccaccctgagcgtgtccccaggcgaaagagctaccctgagctgcaaggccagccagagcgtggaaagcaacgtggcctggtatcagcagaagcccggacaggctcctcgggccctgatctacagcgccagcctgagattcagcggcatccccgccaggtttagcggctctggcagcggcaccgagttcaccctgacaatcagcagcctgcagagcgaggactttgccgtgtattactgccagcagtacaacaactaccccctgaccttcggagccggcaccaagctggagctgaagcctgccgagcctaagagccccgacaagacccacacctgtcccccttgtcctgcccctccagtggctggccctagcgtgttcctgttccccccaaagcccaaggataccctgatgatcgcccggacccccgaagtcacatgcgtggtggtggacgtgagccacgaagaccctgaggtcaagttcaactggtacgtggacggcgtggaggtgcataatgccaagacaaagccgcgggaggagcagtacaacagcacgtaccgtgtggtcagcgtcctcaccgtcctgcaccaggactggctgaatggcaaggagtacaagtgcaaggtctccaacaaagccctcccagcccccatcgagaaaaccatctccaaagccaaagggcagccccgagaaccacaggtgtacaccctgcccccatcccgggatgagctgaccaagaaccaggtgtccctgacctgcctcgtgaagggcttctacccctccgatatcgccgtggaatgggagagcaatggccagcccgagaacaactacaagaccaccccccctgtgctggacagcgacggctcattcttcctgtacagcaagctgacagtggacaagagccggtggcagcagggcaacgtgttcagctgcagcgtgatgcacgaggctctgcacaaccactacacccagaagtccctgagcagcctgagcccaggcaagaagatctacatctgggcccctctggccggcacctgtggcgtgctgctgctgtctctcgtgatcacactgtactgcaagcggggcagaaagaagctgctgtacatcttcaagcagcccttcatgcggcccgtgcagaccacccaggaagaggacggctgctcctgcagattccccgaggaagaagaaggcggctgcgagctgctgcgcgtgaagttttctagaagcgccgacgcccctgcctaccagcagggccagaaccagctgtacaacgagctgaacctgggcagacgggaagagtacgacgtgctggataagcggagaggccgggaccctgagatgggcggcaagcctagaagaaagaacccccaggaaggcctgtataacgaactgcagaaagacaagatggccgaggcctacagcgagatcggaatgaagggcgagcggagaagaggcaagggccacgatggactgtaccagggcctgagcaccgccaccaaggacacctatgacgccctgcacatgcaggctctgccccccaga

SEQ ID NO: 93 - DNA, 2040 bp, synthetic construct
  misc_feature 1..2040: note = construct
  source 1..2040: mol_type = other DNA
atggatttccaggtgcagatcttcagcttcctgctgatctccgccagcgtgatcatgagccgcgagatcgtgatgacacagagccctgccaccctgagcgtgtccccaggcgaaagagctaccctgagctgcaaggccagccagagcgtggaaagcaacgtggcctggtatcagcagaagcccggacaggctcctcgggccctgatctacagcgccagcctgagattcagcggcatccccgccaggtttagcggctctggcagcggcaccgagttcaccctgacaatcagcagcctgcagagcgaggactttgccgtgtattactgccagcagtacaacaactaccccctgaccttcggagccggcaccaagctggagctgaagggcagcaccagcggctccggcaagcctggctctggcgagggcagcacaaagggagaggtgcagctggtggaatctggcggaggactggtgcagcctggcggctctctgagactgtcttgtgccgccagcggcttcaccttcagccggtactggtttagctgggtgcgccaggcccctggcaagggactcgtgtgggtgggagagatcaaccccagcagcagcaccatcaactacgcccccagcctgaaggacaagttcaccatcagcagagacaacgccaagaacaccctgtacctgcagatgaacagcctgcgggccgaggacaccgccgtgtactattgtgccagcctgtactacgactacggcgacgcctacgattactggggccagggcacactggtgactgttagctcccctgccgagcctaagagccccgacaagacccacacctgtcccccttgtcctgcccctccagtggctggccctagcgtgttcctgttccccccaaagcccaaggataccctgatgatcgcccggacccccgaagtcacatgcgtggtggtggacgtgagccacgaagaccctgaggtcaagttcaactggtacgtggacggcgtggaggtgcataatgccaagacaaagccgcgggaggagcagtacaacagcacgtaccgtgtggtcagcgtcctcaccgtcctgcaccaggactggctgaatggcaaggagtacaagtgcaaggtctccaacaaagccctcccagcccccatcgagaaaaccatctccaaagccaaagggcagccccgagaaccacaggtgtacaccctgcccccatcccgggatgagctgaccaagaaccaggtgtccctgacctgcctcgtgaagggcttctacccctccgatatcgccgtggaatgggagagcaatggccagcccgagaacaactacaagaccaccccccctgtgctggacagcgacggctcattcttcctgtacagcaagctgacagtggacaagagccggtggcagcagggcaacgtgttcagctgcagcgtgatgcacgaggctctgcacaaccactacacccagaagtccctgagcagcctgagcccaggcaagaagatctacatctgggcccctctggccggcacctgtggcgtgctgctgctgtctctcgtgatcacactgtactgcaagcggggcagaaagaagctgctgtacatcttcaagcagcccttcatgcggcccgtgcagaccacccaggaagaggacggctgctcctgcagattccccgaggaagaagaaggcggctgcgagctgctgcgcgtgaagttttctagaagcgccgacgcccctgcctaccagcagggccagaaccagctgtacaacgagctgaacctgggcagacgggaagagtacgacgtgctggataagcggagaggccgggaccctgagatgggcggcaagcctagaagaaagaacccccaggaaggcctgtataacgaactgcagaaagacaagatggccgaggcctacagcgagatcggaatgaagggcgagcggagaagaggcaagggccacgatggactgtaccagggcctgagcaccgccaccaaggacacctatgacgccctgcacatgcaggctctgccccccaga

SEQ ID NO: 94 - DNA, 2040 bp, synthetic construct
  misc_feature 1..2040: note = construct
  source 1..2040: mol_type = other DNA
atggatttccaggtgcagatcttcagcttcctgctgatctccgccagcgtgatcatgagccgcgaagtgcagctggtcgaatctggaggaggcctggttcagcctggtggcagccttaggctctcttgtgcagcctctggctttaccttctcacggtattggttcagctgggtgagacaggctccagggaaaggtctggtgtgggtaggggagataaaccccagcagcagcacgatcaactatgctccgtcactgaaagacaagttcaccatttcccgcgataatgccaagaacactctctacttgcagatgaattcccttcgagccgaggatacagcggtgtactactgcgccagtctgtactacgactatggggacgcatacgactattggggacaaggcacactggtgactgttagctccggcagcaccagcggctccggcaagcctggctctggcgagggcagcacaaagggagagatcgtgatgacccagtctcctgctaccctgagcgtttctcccggtgaaagggccacactcagctgcaaagcctctcaaagcgtggagagcaatgtcgcctggtatcagcagaaacctggccaagctccgagagcactgatctattccgcgtcattgcgcttttccggcataccagcacggtttagtggctcagggagtgggactgagttcactctgacgattagctcccttcagtcagaggatttcgccgtgtactactgtcagcagtacaacaactatcccctcacattcggagctggaaccaagctggaactgaagcctgccgagcctaagagccccgacaagacccacacctgtcccccttgtcctgcccctccagtggctggccctagcgtgttcctgttccccccaaagcccaaggataccctgatgatcgcccggacccccgaagtcacatgcgtggtggtggacgtgagccacgaagaccctgaggtcaagttcaactggtacgtggacggcgtggaggtgcataatgccaagacaaagccgcgggaggagcagtacaacagcacgtaccgtgtggtcagcgtcctcaccgtcctgcaccaggactggctgaatggcaaggagtacaagtgcaaggtctccaacaaagccctcccagcccccatcgagaaaaccatctccaaagccaaagggcagccccgagaaccacaggtgtacaccctgcccccatcccgggatgagctgaccaagaaccaggtgtccctgacctgcctcgtgaagggcttctacccctccgatatcgccgtggaatgggagagcaatggccagcccgagaacaactacaagaccaccccccctgtgctggacagcgacggctcattcttcctgtacagcaagctgacagtggacaagagccggtggcagcagggcaacgtgttcagctgcagcgtgatgcacgaggctctgcacaaccactacacccagaagtccctgagcagcctgagcccaggcaagaagatctacatctgggcccctctggccggcacctgtggcgtgctgctgctgtctctcgtgatcacactgtactgcaagcggggcagaaagaagctgctgtacatcttcaagcagcccttcatgcggcccgtgcagaccacccaggaagaggacggctgctcctgcagattccccgaggaagaagaaggcggctgcgagctgctgcgcgtgaagttttctagaagcgccgacgcccctgcctaccagcagggccagaaccagctgtacaacgagctgaacctgggcagacgggaagagtacgacgtgctggataagcggagaggccgggaccctgagatgggcggcaagcctagaagaaagaacccccaggaaggcctgtataacgaactgcagaaagacaagatggccgaggcctacagcgagatcggaatgaagggcgagcggagaagaggcaagggccacgatggactgtaccagggcctgagcaccgccaccaaggacacctatgacgccctgcacatgcaggctctgccccccaga